European Patent Specification EP 3 894 600 B1, published January 4, 2023. Title: METHOD FOR QUANTIFYING A GENOMIC REARRANGEMENT. Applicant: Inivata Ltd. The sequence listing filed with the application follows.

SEQUENCE LISTING (9 sequences)

SEQ ID NO: 1 - DNA, 34 bp, Homo sapien
gaagttcctatactttctagagaataggaacttc

SEQ ID NO: 2 - DNA, 108 bp, Homo sapien
ttaattaaatgtttttcaaatccattcacctgaatgtctaagcttggcaggaagttcctatactttctagagaataggaacttcggaataggaacttcatatggtgcc

SEQ ID NO: 3 - DNA, 68 bp, Homo sapien
aggaagttcctatactttctagagaataggaacttcggaataggaacttcatatggtgccatccctca

SEQ ID NO: 4 - DNA, 499 bp, Homo sapien
cgccaaggtcacagctgctgccaagagagccttgggcgtttcccacctcatggacaatgcagactaggatgtttttagacccaaagacagagtgctgtttctatcccggtgctgtctctaatttgctatgtaactttggacaagtccccttccctctaggattcagggtcctgaagtagaaggtcaaagggccaccctgcctggggcctcagtttctgcatcagattcatagaaggcaccttacatgctattgtcatgtatattttctgtatttattattttttgcagaaagagcacttcaaataatttacagaaccagaatttaaggtggagatgacatttaatggatcctgcagtagtgtttgcacatggaagtccaaaaacctgaaaggaatatttcagttcagagtagtagctgcaaataatctagggtttggtgaatatagtggaatcagtgagaatattatattagttggaggtatgttaccatgtctgtcta

SEQ ID NO: 5 - DNA, 104 bp, Homo sapien
ttacatgctattgtcatgtatattttctgtatttattattttttgcagaaagagcacttcaaataatttacagaaccagaatttaaggtggaagatgacattta

SEQ ID NO: 6 - DNA, 110 bp, Homo sapien
ccctgcctggggcctcagtttctgcatcagattcatagaaggcaccttacatgctattgtcatgtatattttctgtatttattattttttgcagaaagagcacttcaaat

SEQ ID NO: 7 - DNA, 499 bp, Homo sapien; identical to SEQ ID NO: 4

SEQ ID NO: 8 - DNA, 499 bp, Homo sapien; identical to SEQ ID NO: 4

SEQ ID NO: 9 - DNA, 34 bp, Homo sapien; identical to SEQ ID NO: 1